European Patent Specification EP 3 636 275 B1, published August 9, 2023. Title: Pharmaceutical composition for preventing or treating angiogenic diseases comprising collagen type and pigemented epithelium derived factor peptide. Applicant: inje university industry-academic cooperation foundation. The sequence listing filed with the application follows.

SEQUENCE LISTING (1 sequence)

SEQ ID NO: 1 - protein, 34 aa, pigemented epithelium derived factor peptide
DPFFKVPVNKLAAAVSNFGYDLYRVRSSTSPTTN